European Patent Specification EP 3 927 831 B1, published November 12, 2025. Title: Method of producing a binder-toxin fusion protein in a plant cell or a whole plant. Applicant: ATB Therapeutics. The sequence listing filed with the application follows.

SEQUENCE LISTING (18 sequences)

SEQ ID NO: 1 - protein, 474 aa, artificial sequence
  recombinant sequence
QIVLSQSPAILSASPGEKVTMTCRASSSVSYIHWFQQKPGSSPKPWIYATSNLASGVPVRFSGSGSGTSYSLTISRVEAEDAATYYCQQWTSNPPTFGGGTKLEIKGGGGSGGGGSGGGGSQVQLQQPGAELVKPGASVKMSCKASGYTFTSYNMHWVKQTPGRGLEWIGAIYPGNGDTSYNQKFKGKATLTADKSSSTAYMQLSSLTSEDSAVYYCARSTYYGGDWYFNVWGAGTTVTVSAEPKSCDKTHTCPPCPAPELLGGPSVFLFPPKPKDTLMISRTPEVTCVVVDVSHEDPEVKFNWYVDGVEVHNAKTKPREEQYNSTYRVVSVLTVLHQDWLNGKEYKCKVSNKALPAPIEKTISKAKGQPREPQVYTLPPSRDELTKNQVSLTCLVKGFYPSDIAVEWESNGQPENNYKTTPPVLDSDGSFFLYSKLTVDKSRWQQGNVFSCSVMHEALHNHYTQKSLSLSPGK

SEQ ID NO: 2 - protein, 716 aa, artificial sequence
  recombinant sequence
QIVLSQSPAILSASPGEKVTMTCRASSSVSYIHWFQQKPGSSPKPWIYATSNLASGVPVRFSGSGSGTSYSLTISRVEAEDAATYYCQQWTSNPPTFGGGTKLEIKGGGGSGGGGSGGGGSQVQLQQPGAELVKPGASVKMSCKASGYTFTSYNMHWVKQTPGRGLEWIGAIYPGNGDTSYNQKFKGKATLTADKSSSTAYMQLSSLTSEDSAVYYCARSTYYGGDWYFNVWGAGTTVTVSAEPKSCDKTHTCPPCPAPELLGGPSVFLFPPKPKDTLMISRTPEVTCVVVDVSHEDPEVKFNWYVDGVEVHNAKTKPREEQYNSTYRVVSVLTVLHQDWLNGKEYKCKVSNKALPAPIEKTISKAKGQPREPQVYTLPPSRDELTKNQVSLTCLVKGFYPSDIAVEWESNGQPENNYKTTPPVLDSDGSFFLYSKLTVDKSRWQQGNVFSCSVMHEALHNHYTQKSLSLSPGKRHRRHRRRKRSLDTSIIGGHEAKPHSRPYMAYLMIWDQKSLKRCGGFLIRDDFVLTAAHCWGSSINVTLGAHNIKEQEPTQQFIPVKRPIPHPAYNPKNFSNDIMLLQLERKAKRTRAVQPLRLPSNKAQVKPGQTCSVAGWGQTAPLGKHSHTLQEVKMTVQEDRKCESDLRHYYDSTIELCVGDPEIKKTSFKGDSGGPLVCNKVAQGIVSYGRNNGMPPRACTKVSSFVHWIKKTMKRY

SEQ ID NO: 3 - protein, 703 aa, artificial sequence
  recombinant sequence
QIVLSQSPAILSASPGEKVTMTCRASSSVSYIHWFQQKPGSSPKPWIYATSNLASGVPVRFSGSGSGTSYSLTISRVEAEDAATYYCQQWTSNPPTFGGGTKLEIKGGGGSGGGGSGGGGSQVQLQQPGAELVKPGASVKMSCKASGYTFTSYNMHWVKQTPGRGLEWIGAIYPGNGDTSYNQKFKGKATLTADKSSSTAYMQLSSLTSEDSAVYYCARSTYYGGDWYFNVWGAGTTVTVSAEPKSCDKTHTCPPCPAPELLGGPSVFLFPPKPKDTLMISRTPEVTCVVVDVSHEDPEVKFNWYVDGVEVHNAKTKPREEQYNSTYRVVSVLTVLHQDWLNGKEYKCKVSNKALPAPIEKTISKAKGQPREPQVYTLPPSRDELTKNQVSLTCLVKGFYPSDIAVEWESNGQPENNYKTTPPVLDSDGSFFLYSKLTVDKSRWQQGNVFSCSVMHEALHNHYTQKSLSLSPGKGEIIGGHEAKPHSRPYMAYLMIWDQKSLKRCGGFLIRDDFVLTAAHCWGSSINVTLGAHNIKEQEPTQQFIPVKRPIPHPAYNPKNFSNDIMLLQLERKAKRTRAVQPLRLPSNKAQVKPGQTCSVAGWGQTAPLGKHSHTLQEVKMTVQEDRKCESDLRHYYDSTIELCVGDPEIKKTSFKGDSGGPLVCNKVAQGIVSYGRNNGMPPRACTKVSSFVHWIKKTMKRY

SEQ ID NO: 4 - protein, 451 aa, artificial sequence
  recombinant sequence
QVQLQQPGAELVKPGASVKMSCKASGYTFTSYNMHWVKQTPGRGLEWIGAIYPGNGDTSYNQKFKGKATLTADKSSSTAYMQLSSLTSEDSAVYYCARSTYYGGDWYFNVWGAGTTVTVSAASTKGPSVFPLAPSSKSTSGGTAALGCLVKDYFPEPVTVSWNSGALTSGVHTFPAVLQSSGLYSLSSVVTVPSSSLGTQTYICNVNHKPSNTKVDKKAEPKSCDKTHTCPPCPAPELLGGPSVFLFPPKPKDTLMISRTPEVTCVVVDVSHEDPEVKFNWYVDGVEVHNAKTKPREEQYNSTYRVVSVLTVLHQDWLNGKEYKCKVSNKALPAPIEKTISKAKGQPREPQVYTLPPSRDELTKNQVSLTCLVKGFYPSDIAVEWESNGQPENNYKTTPPVLDSDGSFFLYSKLTVDKSRWQQGNVFSCSVMHEALHNHYTQKSLSLSPGK

SEQ ID NO: 5 - protein, 213 aa, artificial sequence
  recombinant sequence
QIVLSQSPAILSASPGEKVTMTCRASSSVSYIHWFQQKPGSSPKPWIYATSNLASGVPVRFSGSGSGTSYSLTISRVEAEDAATYYCQQWTSNPPTFGGGTKLEIKRTVAAPSVFIFPPSDEQLKSGTASVVCLLNNFYPREAKVQWKVDNALQSGNSQESVTEQDSKDSTYSLSSTLTLSKADYEKHKVYACEVTHQGLSSPVTKSFNRGEC

SEQ ID NO: 6 - protein, 455 aa, artificial sequence
  recombinant sequence
QIVLSQSPAILSASPGEKVTMTCRASSSVSYIHWFQQKPGSSPKPWIYATSNLASGVPVRFSGSGSGTSYSLTISRVEAEDAATYYCQQWTSNPPTFGGGTKLEIKRTVAAPSVFIFPPSDEQLKSGTASVVCLLNNFYPREAKVQWKVDNALQSGNSQESVTEQDSKDSTYSLSSTLTLSKADYEKHKVYACEVTHQGLSSPVTKSFNRGECHRRRKRSLDTSRHRRIIGGHEAKPHSRPYMAYLMIWDQKSLKRCGGFLIRDDFVLTAAHCWGSSINVTLGAHNIKEQEPTQQFIPVKRPIPHPAYNPKNFSNDIMLLQLERKAKRTRAVQPLRLPSNKAQVKPGQTCSVAGWGQTAPLGKHSHTLQEVKMTVQEDRKCESDLRHYYDSTIELCVGDPEIKKTSFKGDSGGPLVCNKVAQGIVSYGRNNGMPPRACTKVSSFVHWIKKTMKRY

SEQ ID NO: 7 - protein, 693 aa, artificial sequence
  recombinant sequence
QVQLQQPGAELVKPGASVKMSCKASGYTFTSYNMHWVKQTPGRGLEWIGAIYPGNGDTSYNQKFKGKATLTADKSSSTAYMQLSSLTSEDSAVYYCARSTYYGGDWYFNVWGAGTTVTVSAASTKGPSVFPLAPSSKSTSGGTAALGCLVKDYFPEPVTVSWNSGALTSGVHTFPAVLQSSGLYSLSSVVTVPSSSLGTQTYICNVNHKPSNTKVDKKAEPKSCDKTHTCPPCPAPELLGGPSVFLFPPKPKDTLMISRTPEVTCVVVDVSHEDPEVKFNWYVDGVEVHNAKTKPREEQYNSTYRVVSVLTVLHQDWLNGKEYKCKVSNKALPAPIEKTISKAKGQPREPQVYTLPPSRDELTKNQVSLTCLVKGFYPSDIAVEWESNGQPENNYKTTPPVLDSDGSFFLYSKLTVDKSRWQQGNVFSCSVMHEALHNHYTQKSLSLSPGKHRRRKRSLDTSRHRRIIGGHEAKPHSRPYMAYLMIWDQKSLKRCGGFLIRDDFVLTAAHCWGSSINVTLGAHNIKEQEPTQQFIPVKRPIPHPAYNPKNFSNDIMLLQLERKAKRTRAVQPLRLPSNKAQVKPGQTCSVAGWGQTAPLGKHSHTLQEVKMTVQEDRKCESDLRHYYDSTIELCVGDPEIKKTSFKGDSGGPLVCNKVAQGIVSYGRNNGMPPRACTKVSSFVHWIKKTMKRY

SEQ ID NO: 8 - protein, 227 aa, Homo sapiens
IIGGHEAKPHSRPYMAYLMIWDQKSLKRCGGFLIRDDFVLTAAHCWGSSINVTLGAHNIKEQEPTQQFIPVKRPIPHPAYNPKNFSNDIMLLQLERKAKRTRAVQPLRLPSNKAQVKPGQTCSVAGWGQTAPLGKHSHTLQEVKMTVQEDRKCESDLRHYYDSTIELCVGDPEIKKTSFKGDSGGPLVCNKVAQGIVSYGRNNGMPPRACTKVSSFVHWIKKTMKRY

SEQ ID NO: 9 - protein, 9 aa, artificial sequence
  recombinant sequence
YTFTSYNMH

SEQ ID NO: 10 - protein, 14 aa, artificial sequence
  recombinant sequence
WIGAIYPGNGDTSY

SEQ ID NO: 11 - protein, 13 aa, artificial sequence
  recombinant sequence
RSTYYGGDWYFNV

SEQ ID NO: 12 - protein, 7 aa, artificial sequence
  recombinant sequence
SSVSYIH

SEQ ID NO: 13 - protein, 11 aa, artificial sequence
  recombinant sequence
PWIYATSNLAS

SEQ ID NO: 14 - protein, 8 aa, artificial sequence
  recombinant sequence
QQWTSNPP

SEQ ID NO: 15 - protein, 9 aa, artificial sequence
  recombinant sequence
EEQYNSTYR

SEQ ID NO: 16 - protein, 13 aa, artificial sequence
  recombinant sequence
NFSNDIMLLQLER

SEQ ID NO: 17 - protein, 710 aa, artificial sequence
  recombinant sequence
IIGGHEAKPHSRPYMAYLMIWDQKSLKRCGGFLIRDDFVLTAAHCWGSSINVALGAHNIKEQEPTQQFIPVKRPIPHPAYNPKNFANDIMLLQLERKAKRTRAVQPLRLPSNKAQVKPGQTCSVAGWGQTAPLGKHSHTLQEVKMTVQEDRKCESDLRHYYDSTIELCVGDPEIKKTSFKGDSGGPLVCNKVAQGIVSYGRNNGMPPRACTKVSSFVHWIKKTMKRYHRRRKRSLDTSDKTHTCPPCPAPELLGGPSVFLFPPKPKDTLMISRTPEVTCVVVDVSHEDPEVKFNWYVDGVEVHNAKTKPREEQYNSTYRVVSVLTVLHQDWLNGKEYKCKVSNKALPAPIEKTISKAKGQPREPQVYTLPPSRDELTKNQVSLTCLVKGFYPSDIAVEWESNGQPENNYKTTPPVLDSDGSFFLYSKLTVDKSRWQQGNVFSCSVMHEALHNHYTQKSLSLSPGGGGSQIVLSQSPAILSASPGEKVTMTCRASSSVSYIHWFQQKPGSSPKPWIYATSNLASGVPVRFSGSGSGTSYSLTISRVEAEDAATYYCQQWTSNPPTFGGGTKLEIKGGGGSGGGGSGGGGSQVQLQQPGAELVKPGASVKMSCKASGYTFTSYNMHWVKQTPGRGLEWIGAIYPGNGDTSYNQKFKGKATLTADKSSSTAYMQLSSLTSEDSAVYYCARSTYYGGDWYFNVWGAGTTVTVSA

SEQ ID NO: 18 - protein, 11 aa, artificial sequence
  recombinant sequence
HRRRKRSLDTS